European Patent Application EP 4 239 070 A1, published September 6, 2023. Title: METHOD FOR PRODUCING L-AMINO ACID. Applicant: Ajinomoto Co., Inc. The sequence listing filed with the application follows.

SEQUENCE LISTING (25 sequences)

SEQ ID NO: 1 - DNA, 1281 bp, Corynebacterium glutamicum
atgagttcagtttcgctgcaggattttgatgcagagcgaattggtctgttccacgaggacattaaacgcaagtttgatgagctcaagtcaaaaaatctgaagctggatcttactcgcggtaagccttcgtcggagcagttggatttcgctgatgagctgttggcgttgcctggtaagggcgatttcaaggctgcggatggtactgatgtccgtaactatggcgggctggatggcattgttgatattcgtcagatttgggcggatttgctgggtgttcctgtggagcaggtgctggcgggggatgcttcgagcttgaacatcatgtttgatgtgatcagctggtcgtacatttttggtaacaatgattcggttcagccttggtcgaaggaagaaactgttaagtggatttgtcctgttccgggatatgatcgccatttctccatcacggagcgtttcggctttgagatgatttctgtgccaatgaatgaagacggccctgatatggatgctgttgaggaattggtcaaggatccgcaggttaagggcatgtgggttgtgccggtattttctaacccgactggtttcacggtgtcggaggacgtcgcaaagcgtctgagcacgatggaaactgcggcgccggacttccgcgtggtgtgggataacgcttacgccgttcatactctgaccgatgagttccctgaggtcatcgacatcgttgggcttggtgaggcggcgggtaacccgaaccgtttctgggcgttcacttctacttcgaagatcactctcgcgggtgcgggcgtgtccttcttcatgacttctgcggagaaccgtaagtggtactccggtcatgcgggtatccgtggcattggccctaacaaggtcaatcagttggctcatgcgcgttactttggcgatgctgagggagtgcgcgcggtgatgcgtaagcatgctgcgtcgttggctccgaagttcaacaaggttctggagatcctggattctcgccttgctgagtacggtgtcgcgcagtggactgtccctgcgggcggttacttcatttcccttgatgtggttcctggtacggcatctcgtgtggctgagttggctaaggaagccggcattgcgttgacgggtgcgggttcttcttacccgctgcgtcaggatccggagaacaagaacctccgtttggcgccttctctgcctcctgttgaggaacttgaggttgccatggatggcgtggctacgtgtgttttgctggcagctgcggagcactacgctagctag

SEQ ID NO: 2 - protein, 426 aa, Corynebacterium glutamicum
MSSVSLQDFDAERIGLFHEDIKRKFDELKSKNLKLDLTRGKPSSEQLDFADELLALPGKGDFKAADGTDVRNYGGLDGIVDIRQIWADLLGVPVEQVLAGDASSLNIMFDVISWSYIFGNNDSVQPWSKEETVKWICPVPGYDRHFSITERFGFEMISVPMNEDGPDMDAVEELVKDPQVKGMWVVPVFSNPTGFTVSEDVAKRLSTMETAAPDFRVVWDNAYAVHTLTDEFPEVIDIVGLGEAAGNPNRFWAFTSTSKITLAGAGVSFFMTSAENRKWYSGHAGIRGIGPNKVNQLAHARYFGDAEGVRAVMRKHAASLAPKFNKVLEILDSRLAEYGVAQWTVPAGGYFISLDVVPGTASRVAELAKEAGIALTGAGSSYPLRQDPENKNLRLAPSLPPVEELEVAMDGVATCVLLAAAEHYAS

SEQ ID NO: 3 - DNA, 1179 bp, Corynebacterium glutamicum
atgaccatcgacctgcagcgttccacccaaaacctcacccatgaggaaatcttcgaggcacacgagggcggaaagctctccattagttccactcgtccgctccgcgacatgcgcgatctttcccttgcttacaccccaggtgttgctcaggtttgtgaagcaatcaaagaagatccagaggttgcacgcacccacacgggcattggaaacaccgtcgcggttatttccgacggcaccgctgttcttggccttggcgatatcggacctcaggcatcccttcccgtcatggagggcaaggctcagctgttcagctctttcgctggtttgaaggctatccctatcgttttggatgttcacgatgttgacgctttggttgagaccatcgcagccatcgcgccttctttcggtgctatcaacttggaggacatctccgctcctcgttgcttcgaggtggagcgccgcctcatcgagcgtctcgatattccagttatgcacgatgaccagcacggcaccgctgtggttatcctcgctgcgctgcgcaactccctgaagctgctggatcgcaagatcgaagacctcaagattgttatttccggcgcaggcgcagcgggcgttgcagctgtagatatgttgaccaatgctggcgcaaccgacatcgtggttcttgattcccgaggcatcatccacgacagccgtgaggatctttccccagttaaggctgctctcgcggagaagaccaaccctcgtggcatcagcggtggcatcaatgaggctttcaccggcgcggacctgttcatcggcgtgtccggcggcaacatcggcgaggacgctctcaaactcatggcaccacagccaatcctgttcaccctggcgaacccaaccccagagatcgatcctgaactgtctcagaagtacggcgccatcgtcgcgaccggccgctctgacctgcctaaccagatcaacaacgtgctagcgttcccaggcattttcgccggcgctctcgcagccaaggccaagaagatcacccccgagatgaagctcgctgcagcagaggcaatcgccgacatcgcagctgaggacctcgaggtcggccgcatcgtaccgaccgccttggatccccgcgtcgccccagcagtaaaggcagctgtccaggccgtcgccgaagcgcaaaacgcttag

SEQ ID NO: 4 - protein, 392 aa, Corynebacterium glutamicum
MTIDLQRSTQNLTHEEIFEAHEGGKLSISSTRPLRDMRDLSLAYTPGVAQVCEAIKEDPEVARTHTGIGNTVAVISDGTAVLGLGDIGPQASLPVMEGKAQLFSSFAGLKAIPIVLDVHDVDALVETIAAIAPSFGAINLEDISAPRCFEVERRLIERLDIPVMHDDQHGTAVVILAALRNSLKLLDRKIEDLKIVISGAGAAGVAAVDMLTNAGATDIVVLDSRGIIHDSREDLSPVKAALAEKTNPRGISGGINEAFTGADLFIGVSGGNIGEDALKLMAPQPILFTLANPTPEIDPELSQKYGAIVATGRSDLPNQINNVLAFPGIFAGALAAKAKKITPEMKLAAAEAIADIAAEDLEVGRIVPTALDPRVAPAVKAAVQAVAEAQNA

SEQ ID NO: 5 - DNA, 1740 bp, Corynebacterium glutamicum
atggcacacagctacgcagaacaattaattgacactttggaagctcaaggtgtgaaacgaatttatggtttggtgggtgacagccttaatccgatcgtggatgctgtccgccaatcagatattgagtgggtgcacgttagaaatgaggaagcggcggcgtttgcagctggtgcggaatcgttgatcactggggagctggcagtatgtgctgcttcttgtggtcctggaaacacacacctgattcagggtctttatgattcgcatcgaaatggtgcgaaggtgttggccatcgctagccatattccgagtgcccagattggttcgacgttcttccaggaaacgcatccggagattttgtttaaggaatgctctggttactgcgagatggtgaatggtggtgagcagggtgaacgcattttgcatcacgcgattcagtccaccatggcgggtaaaggtgtgtcggtggtagtgattcctggcgatatcgctaaggaagacgcaggtgacggcacttattccaattccactatttcctcgggcactcctgtggtgttcccggatcctactgaggctgcagcgctggtggaggcgattaacaacgctaagtctgtcactttgttctgcggcgcgggtgtgaagaatgctcgcgcgcaggtgttggagttggcggagaagattaaatcaccaatcgggcatgcgctgggtggtaagcagtacatccagcatgagaatccgtttgaggtcggcatgtctggcctgcttggttacggcgcctgcgtggatgcgtccaatgaggcggatctgctgattctgttgggtacggatttcccttattctgatttccttcctaaagataacgttgcccaggtggatatcaacggtgcgcacattggtcgacgtaccacggtgaagtatccggtgactggtgatgttgctgcaacaatcgaaaatattttgcctcatgtgaaggaaaagacagatcgttccttccttgatcggatgctcaaggcacacgagcgtaagttgagctcggtggtggagacgtacacacataacgtcgagaagcatgtgcctattcaccctgaatacgttgcctctattttgaacgagctggcggataaggacgcggtgtttaccgtggacaccggaatgtgcaatgtgtggcatgcgaggtacatcgaaaatccggagggaactcgcgactttgtgggttcattccgccacggcacgatggctaatgcgttgcctcatgcgattggtgcgcaaagtgccgaccggaaccgccaggtgatcgcgatgtgtggcgatggtggtttgggcatgctgctgggtgagcttctgaccgttaagctgcaccaacttccgctgaaggctgtggtgtttaacaacagttctttgggcatggtgaagttggagatgctcgtggagggacagccagaatttggtactgaccatgaggaagtgaatttcgcagagattgcggcggctgcgggtatcaaatcggtacgcatcaccgatccgaagaaagttcgcgagcagctagctgaggcattggcatatcctggacctgtactgatcgatatcgtcacggatcctaatgcgctgtcgatcccaccaaccatcacgtgggaacaggtcatgggattcagcaaggcggccacccgaaccgtctttggtggaggagtaggagcgatgatcgatctggcccgttcgaacataaggaatattcctactccatga

SEQ ID NO: 6 - protein, 579 aa, Corynebacterium glutamicum
MAHSYAEQLIDTLEAQGVKRIYGLVGDSLNPIVDAVRQSDIEWVHVRNEEAAAFAAGAESLITGELAVCAASCGPGNTHLIQGLYDSHRNGAKVLAIASHIPSAQIGSTFFQETHPEILFKECSGYCEMVNGGEQGERILHHAIQSTMAGKGVSVVVIPGDIAKEDAGDGTYSNSTISSGTPVVFPDPTEAAALVEAINNAKSVTLFCGAGVKNARAQVLELAEKIKSPIGHALGGKQYIQHENPFEVGMSGLLGYGACVDASNEADLLILLGTDFPYSDFLPKDNVAQVDINGAHIGRRTTVKYPVTGDVAATIENILPHVKEKTDRSFLDRMLKAHERKLSSVVETYTHNVEKHVPIHPEYVASILNELADKDAVFTVDTGMCNVWHARYIENPEGTRDFVGSFRHGTMANALPHAIGAQSADRNRQVIAMCGDGGLGMLLGELLTVKLHQLPLKAVVFNNSSLGMVKLEMLVEGQPEFGTDHEEVNFAEIAAAAGIKSVRITDPKKVREQLAEALAYPGPVLIDIVTDPNALSIPPTITWEQVMGFSKAATRTVFGGGVGAMIDLARSNIRNIPTP

SEQ ID NO: 7 - DNA, 1194 bp, Corynebacterium glutamicum
atggcattggcacttgttttgaactccggttcatcttccatcaaattccagctggtcaaccccgaaaactctgccatcgacgagccatatgtttctggtcttgtggagcagattggtgagccaaacggccgcatcgtactcaaagtagagggtgaaaaatacaccctagagacacccatcgcagatcactccgaaggcctaaacctggcgttcgatctcatggaccagcacaactgtggtccttcccaactggaaatcaccgcagttggacaccgcgtggtccacggtggaatcttgttctctgcgccggaactcatcactgatgaaatcgttgaaatgatccgcgatctcattccactcgcaccactgcacaaccctgcaaacgttgacggcattgatgttgctcgaaaaattctccccgatgtcccacacgtagctgtctttgacaccggtttcttccactcacttccaccagcagctgcactgtatgccatcaacaaggatgtcgcagctgaacacggaatcaggcgctatggtttccacggtacctcccacgaatttgtgtccaagcgcgtggtggaaattttggaaaagcccaccgaagacatcaacaccatcaccttccacctgggcaacggcgcatccatggctgctgttcaaggcggccgtgcggtagatacttccatgggtatgacacctctcgcgggacttgtcatgggtacccgaagcggtgacattgatccaggtgtcgttttccatctctcacgcaccgctggcatgagcatcgatgagatcgataatctgctgaacaaaaagtcgggtgtaaagggactttccggagtcaatgatttccgtgaactgcgggaaatgatcgacaacaatgatcaagatgcctggtccgcgtacaacatttacatacaccaactccgccgctacctcggttcctacatggtggcactgggacgggtagacaccatcgtgttcaccgccggtgttggtgaaaatgcccagtttgtccgtgaggatgccttggcaggtttggaaatgtacggcatcgaaatcgatccggagcgcaacgcactgccaaacgatggtcctagattgatttccaccgatgcctccaaggtgaaggtgtttgttattccaactaatgaagagttggctatcgctaggtacgcggtgaagttcgcttag

SEQ ID NO: 8 - protein, 397 aa, Corynebacterium glutamicum
MALALVLNSGSSSIKFQLVNPENSAIDEPYVSGLVEQIGEPNGRIVLKVEGEKYTLETPIADHSEGLNLAFDLMDQHNCGPSQLEITAVGHRVVHGGILFSAPELITDEIVEMIRDLIPLAPLHNPANVDGIDVARKILPDVPHVAVFDTGFFHSLPPAAALYAINKDVAAEHGIRRYGFHGTSHEFVSKRVVEILEKPTEDINTITFHLGNGASMAAVQGGRAVDTSMGMTPLAGLVMGTRSGDIDPGVVFHLSRTAGMSIDEIDNLLNKKSGVKGLSGVNDFRELREMIDNNDQDAWSAYNIYIHQLRRYLGSYMVALGRVDTIVFTAGVGENAQFVREDALAGLEMYGIEIDPERNALPNDGPRLISTDASKVKVFVIPTNEELAIARYAVKFA

SEQ ID NO: 9 - DNA, 1203 bp, Escherichia coli
atgtcgagtaagttagtactggttctgaactgcggtagttcttcactgaaatttgccatcatcgatgcagtaaatggtgaagagtacctttctggtttagccgaatgtttccacctgcccgaagcacgtatcaaatggaaaatggacggcaataaacaggaagcggctttaggtgcaggcgccgctcacagcgaagcgctcaactttatcgttaatactattctggcacaaaaaccagaactgtctgcgcagctgactgctatcggtcaccgtatcgtacacggcggcgaaaagtataccagctccgtagtgatcgatgagtctgttattcagggtatcaaagatgcagcttcttttgcaccgctgcacaacccggctcacctgatcggtatcgaagaagctctgaaatctttcccacagctgaaagacaaaaacgttgctgtatttgacaccgcgttccaccagactatgccggaagagtcttacctctacgccctgccttacaacctgtacaaagagcacggcatccgtcgttacggcgcgcacggcaccagccacttctatgtaacccaggaagcggcaaaaatgctgaacaaaccggtagaagaactgaacatcatcacctgccacctgggcaacggtggttccgtttctgctatccgcaacggtaaatgcgttgacacctctatgggcctgaccccgctggaaggtctggtcatgggtacccgttctggtgatatcgatccggcgatcatcttccacctgcacgacaccctgggcatgagcgttgacgcaatcaacaaactgctgaccaaagagtctggcctgctgggtctgaccgaagtgaccagcgactgccgctatgttgaagacaactacgcgacgaaagaagacgcgaagcgcgcaatggacgtttactgccaccgcctggcgaaatacatcggtgcctacactgcgctgatggatggtcgtctggacgctgttgtattcactggtggtatcggtgaaaatgccgcaatggttcgtgaactgtctctgggcaaactgggcgtgctgggctttgaagttgatcatgaacgcaacctggctgcacgtttcggcaaatctggtttcatcaacaaagaaggtacccgtcctgcggtggttatcccaaccaacgaagaactggttatcgcgcaagacgcgagccgcctgactgcctga

SEQ ID NO: 10 - protein, 400 aa, Escherichia coli
MSSKLVLVLNCGSSSLKFAIIDAVNGEEYLSGLAECFHLPEARIKWKMDGNKQEAALGAGAAHSEALNFIVNTILAQKPELSAQLTAIGHRIVHGGEKYTSSVVIDESVIQGIKDAASFAPLHNPAHLIGIEEALKSFPQLKDKNVAVFDTAFHQTMPEESYLYALPYNLYKEHGIRRYGAHGTSHFYVTQEAAKMLNKPVEELNIITCHLGNGGSVSAIRNGKCVDTSMGLTPLEGLVMGTRSGDIDPAIIFHLHDTLGMSVDAINKLLTKESGLLGLTEVTSDCRYVEDNYATKEDAKRAMDVYCHRLAKYIGAYTALMDGRLDAVVFTGGIGENAAMVRELSLGKLGVLGFEVDHERNLAARFGKSGFINKEGTRPAVVIPTNEELVIAQDASRLTA

SEQ ID NO: 11 - DNA, 1008 bp, Corynebacterium glutamicum
atgaacctaaagaaccccgaaacgccagaccgtaaccttgctatggagctggtgcgagttacggaagcagctgcactggcttctggacgttgggttggacgtggcatgaagaatgaaggcgacggtgccgctgttgacgccatgcgccagctcatcaactcagtgaccatgaagggcgtcgttgttatcggcgagggcgaaaaagacgaagctccaatgctgtacaacggcgaagaggtcggaaccggctttggacctgaggttgatatcgcagttgacccagttgacggcaccaccctgatggctgagggtcgccccaacgcaatttccattctcgcagctgcagagcgtggcaccatgtacgatccatcctccgtcttctacatgaagaagatcgccgtgggacctgaggccgcaggcaagatcgacatcgaagctccagttgcccacaacatcaacgcggtggcaaagtccaagggaatcaacccttccgacgtcaccgttgtcgtgcttgaccgtcctcgccacatcgaactgatcgcagacattcgtcgtgcaggcgcaaaggttcgtctcatctccgacggcgacgttgcaggtgcagttgcagcagctcaggattccaactccgtggacatcatgatgggcaccggcggaaccccagaaggcatcatcactgcgtgcgccatgaagtgcatgggtggcgaaatccagggcatcctggccccaatgaacgatttcgagcgccagaaggcacacgacgctggtctggttcttgatcaggttctgcacaccaacgatctggtgagctccgacaactgctacttcgtggcaaccggtgtgaccaacggtgacatgctccgtggcgtttcctaccgcgcaaacggcgcaaccacccgttccctggttatgcgcgcaaagtcaggcaccatccgccacatcgagtctgtccaccagctgtccaagctgcaggaatactccgtggttgactacaccaccgcgacctaa

SEQ ID NO: 12 - protein, 335 aa, Corynebacterium glutamicum
MNLKNPETPDRNLAMELVRVTEAAALASGRWVGRGMKNEGDGAAVDAMRQLINSVTMKGVVVIGEGEKDEAPMLYNGEEVGTGFGPEVDIAVDPVDGTTLMAEGRPNAISILAAAERGTMYDPSSVFYMKKIAVGPEAAGKIDIEAPVAHNINAVAKSKGINPSDVTVVVLDRPRHIELIADIRRAGAKVRLISDGDVAGAVAAAQDSNSVDIMMGTGGTPEGIITACAMKCMGGEIQGILAPMNDFERQKAHDAGLVLDQVLHTNDLVSSDNCYFVATGVTNGDMLRGVSYRANGATTRSLVMRAKSGTIRHIESVHQLSKLQEYSVVDYTTAT

SEQ ID NO: 13 - DNA, 1011 bp, Escherichia coli
atgagacgagaacttgccatcgaattttcccgcgtcaccgaatcagcggcgctggctggctacaaatggttaggacgcggcgataaaaacaccgcggacggcgcggcggtaaacgccatgcgtattatgctcaaccaggtcaacattgacggcaccatcgtcattggtgaaggtgaaatcgacgaagcaccgatgctctacattggtgaaaaagtcggtactggtcgcggcgacgcggtagatattgctgttgatccgattgaaggcacgcgcatgacggcgatgggccaggctaacgcgctggcggtgctggcagtaggcgataaaggctgcttcctcaatgcgccggatatgtatatggagaagctgattgtcgggccgggagccaaaggcaccattgatctgaacctgccgctggcggataacctgcgcaatgtagcggcggcgctcggcaaaccgttgagcgaactgacggtaacgattctggctaaaccacgccacgatgccgttatcgctgaaatgcagcaactcggcgtacgcgtatttgctattccggacggcgacgttgcggcctcaattctcacctgtatgccagacagcgaagttgacgtgctgtacggtattggtggcgcgccggaaggcgtagtttctgcggcggtgatccgcgcattagatggcgacatgaacggtcgtctgctggcgcgtcatgacgtcaaaggcgacaacgaagagaatcgtcgcattggcgagcaggagctggcacgctgcaaagcgatgggcatcgaagccggtaaagtattgcgcctgggcgatatggcgcgcagcgataacgtcatcttctctgccaccggtattaccaaaggcgatctgctggaaggcattagccgcaaaggcaatatcgcgactaccgaaacgctgctgatccgcggcaagtcacgcaccattcgccgcattcagtccatccactatctggatcgcaaagacccggaaatgcaggtgcacatcctctga

SEQ ID NO: 14 - protein, 336 aa, Escherichia coli
MRRELAIEFSRVTESAALAGYKWLGRGDKNTADGAAVNAMRIMLNQVNIDGTIVIGEGEIDEAPMLYIGEKVGTGRGDAVDIAVDPIEGTRMTAMGQANALAVLAVGDKGCFLNAPDMYMEKLIVGPGAKGTIDLNLPLADNLRNVAAALGKPLSELTVTILAKPRHDAVIAEMQQLGVRVFAIPDGDVAASILTCMPDSEVDVLYGIGGAPEGVVSAAVIRALDGDMNGRLLARHDVKGDNEENRRIGEQELARCKAMGIEAGKVLRLGDMARSDNVIFSATGITKGDLLEGISRKGNIATTETLLIRGKSRTIRRIQSIHYLDRKDPEMQVHIL

SEQ ID NO: 15 - DNA, 1602 bp, Corynebacterium glutamicum
atgattttaggcgtacccattcaatatttgctctattcattgtggaattggattgtcgataccggttttgatgtagcaattatcctggtcttggcgtttttgattccacgtatcggccgactggccatgcgtattatcaagcagcgagtggagtctgcagccgatgcggacaccactaagaaccagctcgcgttcgctggcgttggcgtttatatcgcgcaaattgtggcgtttttcatgcttgccgtctccgcgatgcaggcttttggtttctctctcgcgggcgctgcgattccggcaaccattgcgtcagctgccattggtcttggtgcgcagtcgattgttgcggacttcttggccggatttttcatcctgacggaaaagcaattcggcgtgggtgactgggtgcgctttgagggcaacggcatcgttgttgaaggcaccgtcattgagatcaccatgcgcgcgaccaaaattcgcacgattgcacaagagaccgtgatcatcccgaactccacggcgaaagtgtgcatcaacaattctaataactggtcgcgtgcggttgtcgttattccgatccccatgttgggttctgaaaacatcacagatgtcatcgcgcgctctgaagctgcgactcgtcgcgcacttggccaggagaaaatcgcaccggaaatcctcggtgaactcgatgtgcacccagccacggaagtcacaccgccaacggtggtcggcatgccgtggatggtcaccatgcgtttcctcgtgcaagtcaccgccggcaatcaatggctggtcgaacgcgccatccgcacagaaatcatcaacgaattctgggaagaatacggcagcgcaaccactacatcgggaaccctcattgattccttacacgttgagcatgaagagccaaagacctcgcttatcgacgcctccccccaggctcttaaggaaccgaagccggaggctgcggcgacggttgcatcgctagctgcatcgtctaacgacgatgcagacaatgcagacgcctcggcgatcaatgcaggcaatccagagaaggaacttgattccgatgtgctggaacaagaactctccagcgaagaaccggaagaaacagcaaaaccagatcactctctccgaggcttcttccgcactgattactacccaaatcggtggcagaagatcctgtcgtttggcggacgtgtccgcatgagcacttccctgttgttgggtgcgctgctcttgctgtcactatttaaggtcatgactgtggaaccaagtgagaattggcaaaactccagtggatggctgtcaccaagcactgccacctcaactgcggtgaccacctccgaaacttccgcgccagcaagcacgccttcgatgacagtgcccactacggtggaggagaccccaacgatggaatctagcgtcgaaacgcagcaggaaacctcaacccctgcaaccgcaacgccccagcgagccgacaccatcgaaccgaccgaggaagccacgtcgcaggaggaaacgactgcatcgcagacgcagtctccagcagtggaagcaccaaccgcggtccaagaaacagttgcgccgacgtccaccccttag

SEQ ID NO: 16 - protein, 533 aa, Corynebacterium glutamicum
MILGVPIQYLLYSLWNWIVDTGFDVAIILVLAFLIPRIGRLAMRIIKQRVESAADADTTKNQLAFAGVGVYIAQIVAFFMLAVSAMQAFGFSLAGAAIPATIASAAIGLGAQSIVADFLAGFFILTEKQFGVGDWVRFEGNGIVVEGTVIEITMRATKIRTIAQETVIIPNSTAKVCINNSNNWSRAVVVIPIPMLGSENITDVIARSEAATRRALGQEKIAPEILGELDVHPATEVTPPTVVGMPWMVTMRFLVQVTAGNQWLVERAIRTEIINEFWEEYGSATTTSGTLIDSLHVEHEEPKTSLIDASPQALKEPKPEAAATVASLAASSNDDADNADASAINAGNPEKELDSDVLEQELSSEEPEETAKPDHSLRGFFRTDYYPNRWQKILSFGGRVRMSTSLLLGALLLLSLFKVMTVEPSENWQNSSGWLSPSTATSTAVTTSETSAPASTPSMTVPTTVEETPTMESSVETQQETSTPATATPQRADTIEPTEEATSQEETTASQTQSPAVEAPTAVQETVAPTSTP

SEQ ID NO: 17 - DNA, 3063 bp, Corynebacterium glutamicum
atgattttaggcgtacccattcaatatttgctctattcattgtggaattggattgtcgataccggttttgatgtagcaattatcctggtcttggcgtttttgattccacgtatcggccgactggccatgcgtattatcaagcagcgagtggagtctgcagccgatgcggacaccactaagaaccagctcgcgttcgctggcgttggcgtttatatcgcgcaaattgtggcgtttttcatgcttgccgtctccgcgatgcaggcttttggtttctctctcgcgggcgctgcgattccggcaaccattgcgtcagctgccattggtcttggtgcgcagtcgattgttgcggacttcttggccggatttttcatcctgacggaaaagcaattcggcgtgggtgactgggtgcgctttgagggcaacggcatcgttgttgaaggcaccgtcattgagatcaccatgcgcgcgaccaaaattcgcacgattgcacaagagaccgtgatcatcccgaactccacggcgaaagtgtgcatcaacaattctaataactggtcgcgtgcggttgtcgttattccgatccccatgttgggttctgaaaacatcacagatgtcatcgcgcgctctgaagctgcgactcgtcgcgcacttggccaggagaaaatcgcaccggaaatcctcggtgaactcgatgtgcacccagccacggaagtcacaccgccaacggtggtcggcatgccgtggatggtcaccatgcgtttcctcgtgcaagtcaccgccggcaatcaatggctggtcgaacgcgccatccgcacagaaatcatcaacgaattctgggaagaatacggcagcgcaaccactacatcgggaaccctcattgattccttacacgttgagcatgaagagccaaagacctcgcttatcgacgcctccccccaggctcttaaggaaccgaagccggaggctgcggcgacggttgcatcgctagctgcatcgtctaacgacgatgcagacaatgcagacgcctcggcgatcaatgcaggcaatccagagaaggaacttgattccgatgtgctggaacaagaactctccagcgaagaaccggaagaaacagcaaaaccagatcactctctccgaggcttcttccgcactgattactacccaaatcggtggcagaagatcctgtcgtttggcggacgtgtccgcatgagcacttccctgttgttgggtgcgctgctcttgctgtcactatttaaggggctcttcctgttttagagtgcattgatcttatggaccaactgccctgaatggataaggcaccgcagaatgtagtggttcaaattacggaaacctagagcaatcccacgcaaatgctccaaccgtccgttgatcgcttcgaccggaccgttggagacaccaacatcgaaatacgccaacacatcaccaagtcgtttaaacaaactacgacccaactgcgcgagttccttattcggccccttcaacacccgaagctgatcaataatggtccgcattttcttcttcgcttcacgcttattacccatctgataacaatcaataatcgcctgatacgcaagccacgcaagctttaacaccccgtagtctttgtcatacgcccacaactgctccaagctttcttgctgacgaggactcaaccacttgtgcgtggtcaacaaggtcttccggtttttatacaacggatcctggcttaaaccacgacgctggtatttctcccgctggaggcgttgccggcaggcggtgagcttgtcaccagcaagccgcacaacatggaatggatccatcacgcgacgagcagaaggaatgagttctttacttgctgtggcgtagccttggaacccatccatggacacgatccgtatctgattgcggaactgttcaccgcgggaaccaagccaggaccgtaaagcatcagcactacgacctgggacgacatctaataaccgggcaggacaccgtgagtcataccgatgcccggtcatatcgacaatcacggtgacaaacccatcaccatgcttagccctattatgtgaccacttatgctcatccaccccaatgacatacactccatcaagatggtgaggatcgttatagaccagctcacggcacatatcgagggctagttggcaggttaaatcccaccctagcccaagtgctttcgcggttgcgtgaacactcatccggtcaatagcaaggcgttgcaaaatccagcgggtgacccggtgggtgacctttttaccgtggtcagcgcagcttagttctgcttggaaatacttttgcttacatgtcgggttggtgcagcggtagcgaggtagacggataaacagtttggtgggaaacccgacgatgggtaaatcaatgagcatccggtgggtgtgatgacgaaacaccccaggttgggagcattctgggcaggtggaggtatagtcgagtgcgtctgcttcgatcagggtgtaatcacctgcatcggaagcgccggtgatggtgagtcctagttccgcagtgcggcagatggtgtcagcgatgatgttgccggtagacttcatgggtagagccttttgttggtgtttggttagcttagatacctaaaccttaaccctgacaaaaggctcgtttattttcgggtctacaccgctagcccaggttctgtgatgtaccccaaaaccggaagggccatttaaggtcatgactgtggaaccaagtgagaattggcaaaactccagtggatggctgtcaccaagcactgccacctcaactgcggtgaccacctccgaaacttccgcgccagcaagcacgccttcgatgacagtgcccactacggtggaggagaccccaacgatggaatctagcgtcgaaacgcagcaggaaacctcaacccctgcaaccgcaacgccccagcgagccgacaccatcgaaccgaccgaggaagccacgtcgcaggaggaaacgactgcatcgcagacgcagtctccagcagtggaagcaccaaccgcggtccaagaaacagttgcgccgacgtccaccccttag

SEQ ID NO: 18 - protein, 423 aa, Corynebacterium glutamicum
MILGVPIQYLLYSLWNWIVDTGFDVAIILVLAFLIPRIGRLAMRIIKQRVESAADADTTKNQLAFAGVGVYIAQIVAFFMLAVSAMQAFGFSLAGAAIPATIASAAIGLGAQSIVADFLAGFFILTEKQFGVGDWVRFEGNGIVVEGTVIEITMRATKIRTIAQETVIIPNSTAKVCINNSNNWSRAVVVIPIPMLGSENITDVIARSEAATRRALGQEKIAPEILGELDVHPATEVTPPTVVGMPWMVTMRFLVQVTAGNQWLVERAIRTEIINEFWEEYGSATTTSGTLIDSLHVEHEEPKTSLIDASPQALKEPKPEAAATVASLAASSNDDADNADASAINAGNPEKELDSDVLEQELSSEEPEETAKPDHSLRGFFRTDYYPNRWQKILSFGGRVRMSTSLLLGALLLLSLFKGLFLF

SEQ ID NO: 19 - DNA, 36 bp, Artificial Sequence
  primer
ccaagcttgcatgccatggcattggcacttgttttg

SEQ ID NO: 20 - DNA, 37 bp, Artificial Sequence
  primer
cggtacccggggatcctaagcgaacttcaccgcgtac

SEQ ID NO: 21 - DNA, 35 bp, Artificial Sequence
  primer
ccaagcttgcatgccatttgcgcctgcaacgtagg

SEQ ID NO: 22 - DNA, 36 bp, Artificial Sequence
  primer
aagtgccaatgccataacaggaatgttcctttcgaa

SEQ ID NO: 23 - DNA, 36 bp, Artificial Sequence
  primer
aggaacattcctgttatggcattggcacttgttttg

SEQ ID NO: 24 - DNA, 52 bp, Artificial Sequence
  primer
ccaagcttgcatgcctgcagaggaggattataatgagacgagaacttgccat

SEQ ID NO: 25 - DNA, 36 bp, Artificial Sequence
  primer
cggtacccggggatccggactggaaggctcaatcga